European Patent Specification EP 3 130 664 B1, published May 21, 2025. Title: Coryneform transformant and method of producing 4-hydroxybenzoate using thereof. Applicant: Green Phenol Technology Research Association. The sequence listing filed with the application follows.

SEQUENCE LISTING (63 sequences)

SEQ ID NO: 1 - DNA, 513 bp, Pantoea ananatis
atgacgcaagacccgctccgttcgttacgttcacttaactggctggcgctggacgatgccgcattgacgcaaccgcttcgtgactggctaatggaagaggattccatgacgcgacgctttgaacagcattgccagaaggtcagggtggaacctgtacgtgaggactttatctccgccgatgaactcggcgatgaaggggcattactccctgccgatcagcgtttctggctgcgagaagtcattctctacggggatgaggaaccttggctggcagggcgcacgctggtgccagaaagtaccctcaacggcccggaagcgatgttacagcaactcggtacgcgcccgctggggcgttatctgttctcgtcatcaacgctgacccgcgatttcattgagcctggccgcgttgatgcgctctggggacgccgctcgcgcctgcgactgtcagggaaaccgctgctgttaacggaactgtttttaccggcttcgccgctctatcgtgatcaaggttaa

SEQ ID NO: 2 - DNA, 519 bp, Providencia rustigianii
atgcatgaaacaatttttacccatcatcccattgattggctaaacgaggatgatgagtcagttcctaacagtgtactagattggctgcaagagcgtggttcaatgactaaacggttcgagcagcattgccaaaaagtcacggtaattccctatttagagcgctatatcactccagagatgctgagcgctgatgaagccgagcgtttacccgaaagtcaacgttactggttgcgagaagtcattatgtatggggataatattccgtggttgataggcagaacattgatccctgaagagaccctcaccaacgatgataaaaagctggtggacattggtcgtgtgccattagggcgttacctttttagtcatgatagtcttacccgagattatattgatattggcaccagtgcggatcgttgggtgcgacgttctctgctgagattatctcaaaagcccttattattaactgaaatatttttacctgaatcacctgcatatagataactatctaacataatc

SEQ ID NO: 3 - DNA, 537 bp, Providencia stuartii
atggatgaaacgctttttatctctcacccgataacatggctatcagaagatgatgaccttgttcctgaaaatgttttagattggctacatgaactagggtcgatgacaaaacgcttagagcagcattgccaacgtgtcacggttgttccttatacgcaacgttatgtgactcaagaggcattgagcgaagaagaagcggcgtgtttacctgtcagtgaatattattggttacgtgaagtcattatgtatggtgataatattccatggttacttggacgaacgttaattccacaggagacattgactggtgaagaccggaaacttattgatatcggtgctgtaccgttagggcgttatctctttagccatgataatctttcccgtgattatattcatatagggcagcaaaatttgcgatggatccgccgctctctattaagattatctgaaaaacctttattattaaccgaactgtttttacctgaatcacctgcatataaaagataaaaaataaaaggagcacaacaaatggaggga

SEQ ID NO: 4 - DNA, 539 bp, Providencia sneebia
atggatgatacgctttttacctctcacccgataacatggttatcagagactgataatgttattcctgaaaatatgttaagttggttacaagaactcgggtcaatgacaaagcgcttagaacaatattgccagtctttgactgtcaccccttatgtgcaaaaatatgtttccagaaacatgctgagtgatgatgaagctcaatgtttacctgaaagctcaagttattggctaagagaagtgattatctatggggataatatcccttggttgctagggcgaacgctaattccgcaagaaacattgagtggcgatgaccaaagaattgtcgatattggtacgctgcctttaggccgttatctatttagtcatgataatctgactcgtgattatattcatattgggcaacaggagcagcgatggctgcgtcgttcgcgattaaggctatcgaataatcctttattattaactgaattgtttttacctgaatcacctgcatataaaagataaaaaataaaaggagcatgacaagtgaagggaag

SEQ ID NO: 5 - DNA, 504 bp, Providencia rettgeri
atggatgaaacgctttttacttctcagccgattcactggctggcggagaacgataaaatagtgcctgccaatgtattagattggctattagagctcggctccatgacaaaacgttttgagcagcatagccagcaagttaccgtgataccttatttagagcgctatataacacaagataagctgagtgcagatgaaatgctgtctttacctgaaagccaacgttattgggtcagagaagttgtcatgtatggagatggtatcccttggttactgggccgaacgataatccctgaagaaacactgactgatgatgaccagcaactggtagatattgggagaatgccgttagggcgttatttatttagccgtgacagcttaactcgagattatattcatattggttcttgcgcaaaccgttgggtacgttgttctcggttaagattatcggataaacccttactattaacagaaatatttttacctgaatcacctgcatatcgttaa

SEQ ID NO: 6 - DNA, 505 bp, Providencia alcalifaciens
atgcatgaaacgatttttacctctcatcctataagttggttcgtagaaggcgaagagagtgttcctgaaaatgtattaggttggttgcaagagcaaaggtcgatgaccaaacggtttgagcagcattgtcagaaagtgacggtgataccttatttagaacgctatatctcactggatatgctcaccaccgacgaacaaaaatgcttaccaattagtgagcgttattggctacgggaagtgattatgtatggggataatatcccttggttgattggcagaacgctgatcccagaagagacgctcaccgataatgacaaaaaattagtcgagcttgggcgagtcccattagggcgctatctctttagtcatgaacacctaacccgagattatattgaaatgggcaccagtgctgaccgctgggttcgccgttccttacttagactgtcccaaaaaccattattattaaccgaaatatttttacctgaatcacctgcatatagataac

SEQ ID NO: 7 - DNA, 542 bp, Providencia burhodogranariea
atggatgaaacgctttttacctctcacccgataacgtggctaccagaggccgatgaccttgttcctgataatattttagactggttgcatgagcttgggtcaatgacaaaacgtttagagcagcactgccagtgtgttaccgttatcccttgtgcgcagcgatatgtgactaaagaagctctcagtgatgatgaaactcaatgtttaccggtgagtgagtactattggttacgggaggttattatgtatggtgataatattccctggttactcggccgaacactaattccgcaagaaacattgaccggtgaagaccaaaagctcattgatattggtgctgtaccattagggcgttatctatttagtcatgataatcttacccgggattatattcatatagggcagcaaaattctcgatggctccgtcgctctcgattaaggttatcaaacaaaccgttattattaactgaattatttttacctgaatcacctgcttataaaagataaaaagtaaaaggagcacgacaagtggagggaagtat

SEQ ID NO: 8 - DNA, 498 bp, Escherichia coli
atgtcacaccccgcgttaacgcaactgcgtgcgctgcgctattgtaaagagatccctgccctggatccgcaactgctcgactggctgttgctggaggattccatgacaaaacgttttgaacagcagggaaaaacggtaagcgtgacgatgatccgcgaagggtttgtcgagcagaatgaaatccccgaagaactgccgctgctgccgaaagagtctcgttactggttacgtgaaattttgttatgtgccgatggtgaaccgtggcttgccggtcgtaccgtcgttcctgtgtcaacgttaagcgggccggagctggcgttacaaaaattgggtaaaacgccgttaggacgctatctgttcacatcatcgacattaacccgggactttattgagataggccgtgatgccgggctgtgggggcgacgttcccgcctgcgattaagcggtaaaccgctgttgctaacagaactgtttttaccggcgtcaccgttgtactaa

SEQ ID NO: 9 - DNA, 663 bp, Escherichia fergusonii
atgctgattttgcaacaactggtgcgtcttctggcgcacctttttttatcattttttgcgattgttgcgtttttgttgcgcaatagatcacttaattttgtttccttctcccgtaatctcttttctgcgatacaatgccttcacgttatagaacggagagttcgcatgtcacatcccgcgttaacgcaactgcgtgcgctgcgctattttgctgagattccggcgcttgatcccgcacaactcgactggttattactggaagattccatgaccaaacgttttgagcagcagggaaaaaaggtgagcgtgacagtaatccgcgaaggctttgtcgggcaacaagatgttgccctggagttatcgcagttgccgcaagagcctcgctactggctgcgggaaattttactttgcgcagatggtgaaccctggcttgcggggcgcactgtggtgccagaatcaacgttatctggccctgaactggcattacaaaaactgggtaagaccccgttggggcgctacctgtttacatcatcaacgttgagccgtgattttattgagattggtcgtgatgcagagctatgggggcggcgttcacgtctgcggttaagcggtaagcccctgatgcttactgaactgtttttgcctgcatcaccgttgtactaa

SEQ ID NO: 10 - DNA, 554 bp, Pseudoalteromonas piscicida
atgcctttgcaattacccttagagctcccttggctgaagaacacacagttggtggatgttgagccagcactttctccttatttactagaggctcaatctctaaccgcaaaattgaaagaaacttgtgaaaggttttctgtgactgtgcttgctaatgagttcaggagcgctcctgaagcgttacgtacggatctttctgaacaggtttggtgccgagaagtaacgttaaattgtaacggtaaagcagctgtatttggacaaagttggctcaatgaggacgcatgtactgtcggaatggatgcaattggtgagacacctttgggtgagttactgtttactgattcaaattggcagcgcggaacccttgagtttcttcgtttatctactgccgactatccggcgctgattgaacttattgcacccacaactggcgtcgccccagagcgtttatttgctagaagaagctggtttaaaaacggcaaagcaaagattttagtttgtgaagtctttatatcggaaagcttttatgattgaccaccagaaatggcaggctt

SEQ ID NO: 11 - DNA, 546 bp, Pseudoalteromonas haloplanktis
atgattactttccctgtttcattatctgctgattggcagagtaccgctcaagtaactggcttatctaacgctgagaaagagtggttatttgaaccgcattctttaacggctaaattaaaaagtcagtctcagcgttttgctgtaaaagtgttgagtgagcaaaaagtagacctttcgcaatcacagcaaacgctattaagtgagcaggtaagtacagtacttaaccgtgaagtgttactgttgtgtgatgaacaaccgattgtttatgctcaaagttggttgccagtaacaagcaataatacaaacaatcagctgcacaatatgggagaacgcccgttaggtgatgttatctttcaagatcctgcgttaaggcgcactgatattgaaattgctcgctttgatgataatcacccattgcaatcactggtgagcgaacttaatttaccgaatcgctctttactgggcagacgcagcgtattttctttacataactacaaatttttagtttgtgaagtttttttaccaggagcgtatttgtactcatga

SEQ ID NO: 12 - DNA, 534 bp, Cronobacter sakazakii
atgtcccatcccgcgctgagacaactgcgcgcgttgtccttttttgacgatatcagcacgcttgatagttcgctgctcgactggctgatgctggaagattccatgacccgccgtttcgaaggcttttgcgagcgcgtgacggtcgacatgctgtttgagggctttgtcggccccgaggcgctggaggaagagggcgagtttttgcctgatgagccgcgctactggctgcgcgaaatcctgctgtgcggcgacggcgtgccgtggctggttgggcgcacgctggtgccggagtctacactttgtgggccggagctggcgttgcagcagctcggtaccacgccgctgggccgttatctgtttacctcatccaccctcacgcgtgattttatccagccgggccgcagcgacgaactctggggacgccgctctctgctgaggctttccggcaaaccgctgctgctgactgaactgtttttacctgcatcacccttgtacggagaggaaaaataatggagtggagcctgacgcagaata

SEQ ID NO: 13 - DNA, 498 bp, Citrobacter youngae
atgccacaccctgcgttaacgcaactgcgtgcgctgcgttattttgatgagatcccggcgctggacccgcagctgctcgactggttgttactggaagattcgatgaccaaacgttttgagcagcagggaaaacaagtcaccgttacgttgattcgcgaagcgttcgttgggcaaaatgaggtggctgaagaactgatgctgctgcctaaagaatcccgctactggttacgcgaaatcctgttatgcgcggatggtgagccctggcttgccgggcgtaccgtggtgcctgaatcaaccctgtgcggccctgaactggccttacaaaatctggggaaaaccccgctcggacgctacctgtttacgtcatcgacattgacccgagattttattgagattggccgcgatgcagcgctgtgggggcgacgttcccgcctgcggctgagcggtaagccattgatgcttaccgagctttttctacctgcatcgccgttgtactga

SEQ ID NO: 14 - DNA, 498 bp, Citrobacter koseri
atgtcacaccctgcgttaacgcaactgcgtgcgctgcgctattttaaagagattcctgcgctggattcccggttgctcgactggttacttctggaagattccatgaccaaacgttttgagcaagaagggaaacgggtaagcgtgacattgcttcgggaagcgtttgttggtccacatgaagtggctgaagaggtggcgctgctaccggtcgaatcccgctactggttacgtgaaattttgttatgtgcagacggcgaaccctggcttgccgggcgtaccgtcgtgcctgaatcaacgttgtgcggccctgagctggccttacaaaatctgggaaaaacgccgttagggcgctacctgtttacatcatcaacgttgacccgagattttattgagattggtcgtgatgccgcactgtgggggcgtcgttcccgcctgcgtctgagcggtaagccgctgatgcttaccgagctgtttttgcccgcatcaccgttgtattaa

SEQ ID NO: 15 - DNA, 498 bp, Enterobacter aerogenes
atgccacatcctgcgcttacgcaactgcgtgcgctgcgctattttgccgccatacccgagctggacgcgccgctgcgcgactggctgttgctggaagactcaatgaccaaacgctttgagcaacaagggaaaaaggtcaccgtgaccatgattaacgaaggtttcgtcgggcgcgacgcgctggcgggcgaagaagccctgctgccggaagaggcgcggtattggctgcgggagatcattctttgcgccgatggcgaaccctggcttgccggtcgtactctcgtgccggaatcgacgctatgcggcccggaattagccctgcagcagttggggcagacgccgctgggccggtatctgtttacgtcgtcgacgttaacccgtgattttattgagattggccgtagtgcacagctgtgggggcgacgttcccgtctccggctgagcggcaaaccgctgctgctgacagagctttttctgcctgcatcgccattgtattaa

SEQ ID NO: 16 - DNA, 498 bp, Enterobacter cloacae
atgtcacaccctgcgctaacgcaactgcgttcgctgcgctatttcgaccaaatacctgcgcttgacccgcagcagcttgactggttgctgctggaagattccatgactaaacgttttgagcaacagggcaagacggttacggtgacgatgattcaggaagggtttgtcacctccgctgacattgccagtgagctgccgctgttaccaaaagaagaacgctactggttgcgtgaaattctgctctgcgcggatggtgagccgtggctcgccggacgaaccgtggtgcctgaatccaccctttccgggcctgagctggcactgcaacggctgggaaacaccccgctcgggcggtaccttttcacctcgtctgaacttacccgggattttattgaaattggacgcgatgccgaactgtggggacgtcgttcccgtcttcgcctgagcggtaaaccgttaatactgacggagctttttttaccggcatcgccgttgtactga

SEQ ID NO: 17 - DNA, 558 bp, Pseudomonas putida
atgtcgtacgaatccccgcaagcagccgctgtcgcgtggctgccgtattcacagctggcgaccgacatcgaccagcccacccttgactggctgttcgacgagggctcgctgacccgccgcctgacccgtctgtccattgatcacttttccgtcaccccgttgttcgagggctggcagccgctgcgcgatgacgaatgccaggcgctgggcatcgctgccggcgccgaaggctgggtgcgcgaagtgtatctgcgcggccatggccaaccttgggtattcgcccgcagcgtggccagccgcagcgccctggaacgtggtggcctggacctggaaaccttgggcagccgctcgctgggcgagctgctgttctgcgaccaggcgttcatccgtcatccactcgaagtgtgcacttatccacaggcctggctgccgtccgaagctgcacatgcggcgctttggggccgccgctcgcgcttcgagcgcaacggcctggacctgctggtggcagaagtgttcctgccggcattgtggcaagcggccaaggaggaaaaccgctga

SEQ ID NO: 18 - DNA, 529 bp, Morganella morganii
atgacacaaacagtgataacaccccccatccgctggtttgataatgcggaaatgatccccgccggggtgctggactggttatcagaattagggtcaatgacgcggcgctttgaacagcactgcaatgaagtgacggtaaaaccgtattgtgaaaaatatatctcccgtgaagcgctgactgaagaagagcagatgcatctgcccggcagtgcacgctactggttacgggaggtggtgttatatggtgacggggttccctggctgaccggccggacagtggtaccggaggagacgctgacaggggaagagcagcagttactgaaaatgggaaatgtgccgctcgggcgctatctctttaccagcggttgtctgacgcgggattatatccgcttcgggctgtcagaaacgcactgggcgcgctgttcgcggctgtgcctggccggtaaaccgcttctgctgactgaagtttttctgccggcctctccggcataccccgcataagtgaatatctcggagaagaataacgtgg

SEQ ID NO: 19 - DNA, 552 bp, Azotobacter vinelandii
atgaccgctgctcccgctttccaatggctcggcgccgaccaactgcatcccgcccccccggccgtcctggccgactggctgttcgacagcggctcgctgacccgccggctgaccgccctttccgccggccgtttcgccgtgacgccgctggccgaaggctggcaggtgctgcgcgacgacgaatgcaccgccctcgacgtggtgccgggcagcaccggctgggtacgcgaggtctacctgctcggcgccgagcggccctgggtgttcgcccgcagcgtggcggcccgcgaggctctggcgggtttctccggcgtactcgccgaactcggccggcggcccctcggcgaactgctgttcagcgacccagccttcgcccgcggcccgctgcaggccacgcactatccgccggactggctgccggccgggatacgctgccccggactctggggacggcgctcccgtttccaccgggaaaccctgagcgtgctggtggcggaagtcttcctgccggagctctggcgctaccagggaatcgacccggacaccctataa

SEQ ID NO: 20 - DNA, 561 bp, Shewanella putrefaciens
atgaatgtgactagcttaagcttcccctatggtgaatctattcaatggttttgtgctgatcgtaccgataaacttcccccgtcaccgctaaaagagtggttactcgccccaggcagcctgacaaaaaaactcaaaacctgctgcaatcagtttgaagtcaaagtcctcggtgaaggccaactcgcccccttcaaagatgaatatcctcagcaaggctctgtttgggttcgtgaagtattgctatgccttgataatgttccttgggtgtttgccagaaccttaatcccactctctttgctgtctgaacgagaagcggattttctcggtttgggttctcgtccccttggcgaattactctttagccaagataactttatccccggcagaatagaagtcgccagctttgatacaggtagtcgtcttgcacacttagctgcaagtttagatcaaagggttgaacatctcctgtggggacgccgtcgctattttcaccacggccaggatgagatgatcgtcagtgaaatatttttacctgcggccgagcgagcaatttgccagtga

SEQ ID NO: 21 - DNA, 671 bp, Cupriavidus taiwanensis
atgagcgcgcagtccgtgcgcggctgcggctggagcccgcacctggctttcgatgcggcgatcccgcccaacctgcggcgctgggttaccggcgatgacggctcgctgacggcgcggctggtggccgcctccgcgcgctttcgcgtggcgcggctgctgcaggcgccgcagcgcccgtttgccgacgaatggcaggcgctgggccagcccgaccgcacccccgcgctgacgcgcgaggtgctgctgatctgcgacgacatccccgccgtgttcgcccataccgtggtgcggctgcgccatgcgcgccgcgactggccgttcctgcgcgggctgggcgaacgcccgctgggcgggcgcctgttcgtcgatccggcggtgcggcgcgagccgttccagtttgcgcggctgctgccgcaccatccgctgcgccaggccctgcaccgcgtgctgccggccatggcggcagtgccgatgctgaccgcgcggcgttcggtgttccggcgcggcggcggcgtcatgctcgtgacagaagtgttcctgccagacctgctgtcgcggccatccccggggaccgaggcggtaccgcatcccaaatatatgcggacgacagaccgaagccctgtttcgacacacactaccgaaaccaagaaagagaccacgagatgaaactg

SEQ ID NO: 22 - DNA, 24 bp, Artificial sequence
  PCR primer
ctctcatatgacgcaagacccgct

SEQ ID NO: 23 - DNA, 33 bp, Artificial sequence
  PCR primer
ctctcatatgttaaccttgatcacgatagagcg

SEQ ID NO: 24 - DNA, 36 bp, Artificial sequece
  PCR primer
ctctcatatgcatgaaacaatttttacccatcatcc

SEQ ID NO: 25 - DNA, 42 bp, Artificial sequence
  PCR primer
ctctcatatggattatgttagatagttatctatatgcaggtg

SEQ ID NO: 26 - DNA, 34 bp, Artificial sequence
  PCR primer
ctctcatatggatgaaacgctttttatctctcac

SEQ ID NO: 27 - DNA, 30 bp, Artificial sequence
  PCR primer
ctctcatatgtccctccatttgttgtgctc

SEQ ID NO: 28 - DNA, 32 bp, Artificial sequence
  PCR primer
ctctcatatggatgatacgctttttacctctc

SEQ ID NO: 29 - DNA, 30 bp, Artificial sequence
  PCR primer
ctctcatatgcttcccttcacttgtcatgc

SEQ ID NO: 30 - DNA, 34 bp, Artificial sequence
  PCR primer
ctctcatatggatgaaacgctttttacttctcag

SEQ ID NO: 31 - DNA, 34 bp, Artificial sequence
  PCR primer
ctctcatatgttaacgatatgcaggtgattcagg

SEQ ID NO: 32 - DNA, 35 bp, Artificial sequence
  PCR primer
ctctcatatgcatgaaacgatttttacctctcatc

SEQ ID NO: 33 - DNA, 35 bp, Artificial sequence
  PCR primer
ctctcatatggttatctatatgcaggtgattcagg

SEQ ID NO: 34 - DNA, 32 bp, Artificial sequence
  PCR primer
ctctcatatggatgaaacgctttttacctctc

SEQ ID NO: 35 - DNA, 30 bp, Artificial sequence
  PCR primer
ctctcatatgatacttccctccacttgtcg

SEQ ID NO: 36 - DNA, 26 bp, Artificial sequence
  PCR primer
ctctcatatgtcacaccccgcgttaa

SEQ ID NO: 37 - DNA, 29 bp, Artificial sequence
  PCR primer
ctctcatatgttagtacaacggtgacgcc

SEQ ID NO: 38 - DNA, 31 bp, Artificial sequence
  PCR primer
ctctcatatgctgattttgcaacaactggtg

SEQ ID NO: 39 - DNA, 31 bp, Artificial sequence
  PCR primer
ctctcatatgttagtacaacggtgatgcagg

SEQ ID NO: 40 - DNA, 31 bp, Artificial sequence
  PCR primer
ctctcatatgcctttgcaattacccttagag

SEQ ID NO: 41 - DNA, 30 bp, Artificial sequence
  PCR primer
ctctcatatgaagcctgccatttctggtgg

SEQ ID NO: 42 - DNA, 36 bp, Artificial sequence
  PCR primer
ctctcatatgattactttccctgtttcattatctgc

SEQ ID NO: 43 - DNA, 33 bp, Artificial sequence
  PCR primer
ctctcatatgtcatgagtacaaatacgctcctg

SEQ ID NO: 44 - DNA, 27 bp, Artificial sequence
  PCR primer
ctctcatatgtcccatcccgcgctgag

SEQ ID NO: 45 - DNA, 30 bp, Artificial sequence
  PCR primer
ctctcatatgtattctgcgtcaggctccac

SEQ ID NO: 46 - DNA, 26 bp, Artificial sequence
  PCR primer
ctctcatatgccacaccctgcgttaa

SEQ ID NO: 47 - DNA, 29 bp, Artificial sequence
  PCR primer
ctctcatatgtcagtacaacggcgatgca

SEQ ID NO: 48 - DNA, 27 bp, Artificial sequence
  PCR primer
ctctcatatgtcacaccctgcgttaac

SEQ ID NO: 49 - DNA, 31 bp, Artificial sequence
  PCR primer
ctctcatatgttaatacaacggtgatgcggg

SEQ ID NO: 50 - DNA, 27 bp, Artificial sequence
  PCR primer
ctctcatatgccacatcctgcgcttac

SEQ ID NO: 51 - DNA, 32 bp, Artificial sequence
  PCR primer
ctctcatatgttaatacaatggcgatgcaggc

SEQ ID NO: 52 - DNA, 26 bp, Artificial sequence
  PCR primer
ctctcatatgtcacaccctgcgctaa

SEQ ID NO: 53 - DNA, 28 bp, Artificial sequence
  PCR primer
ctctcatatgtcagtacaacggcgatgc

SEQ ID NO: 54 - DNA, 25 bp, Artificial sequence
  PCR primer
ctctcatatgtcgtacgaatccccg

SEQ ID NO: 55 - DNA, 29 bp, Artificial sequence
  PCR primer
ctctcatatgtcagcggttttcctccttg

SEQ ID NO: 56 - DNA, 31 bp, Artificial sequence
  PCR primer
ctctcatatgacacaaacagtgataacaccc

SEQ ID NO: 57 - DNA, 30 bp, Artificial sequence
  PCR primer
ctctcatatgccacgttattcttctccgag

SEQ ID NO: 58 - DNA, 23 bp, Artificial sequence
  PCR primer
ctctcatatgaccgctgctcccg

SEQ ID NO: 59 - DNA, 28 bp, Artificial sequence
  PCR primer
ctctcatatgttatagggtgtccgggtc

SEQ ID NO: 60 - DNA, 32 bp, Artificial sequence
  PCR primer
ctctcatatgaatgtgactagcttaagcttcc

SEQ ID NO: 61 - DNA, 29 bp, Artificial sequence
  PCR primer
ctctcatatgtcactggcaaattgctcgc

SEQ ID NO: 62 - DNA, 25 bp, Artificial sequence
  PCR primer
ctctcatatgagcgcgcagtccgtg

SEQ ID NO: 63 - DNA, 30 bp, Artificial sequence
  PCR primer
ctctcatatgcagtttcatctcgtggtctc